European Patent Specification EP 3 433 269 B1, published September 27, 2023. Title: Fusion proteins of PD-1 and 4-1BB. Applicant: Helmholtz Zentrum Muenchen. The sequence listing filed with the application follows.

SEQUENCE LISTING (30 sequences)

SEQ ID NO: 1 - DNA, 495 bp, human
atgcagattcctcaggccccttggcctgtcgtgtgggctgtgctccagctgggatggcggcctggctggtttctggacagccccgacagaccctggaacccccctacattttcccctgccctgctggtcgtgaccgagggcgacaatgccaccttcacctgtagcttcagcaacaccagcgagagcttcgtgctgaactggtacagaatgagccccagcaaccagaccgacaagctggccgccttccccgaggatagatctcagcccggccaggattgccggttcagagtgacccagctgcccaacggccgggacttccacatgtctgtcgtgcgggccagacggaacgacagcggcacatatctgtgcggcgccatcagcctggcccccaaggcccagatcaaagagagcctgagagccgagctgagagtgaccgagagaagggccgaagtgcctaccgcccaccctagcccatctccaagacctgccggccag

SEQ ID NO: 2 - protein, 165 aa, human
MQIPQAPWPVVWAVLQLGWRPGWFLDSPDRPWNPPTFSPALLVVTEGDNATFTCSFSNTSESFVLNWYRMSPSNQTDKLAAFPEDRSQPGQDCRFRVTQLPNGRDFHMSVVRARRNDSGTYLCGAISLAPKAQIKESLRAELRVTERRAEVPTAHPSPSPRPAGQ

SEQ ID NO: 3 - DNA, 129 bp, human
aagcggggcagaaagaagctgctgtacatcttcaagcagcccttcatgcggcccgtgcagaccacccaggaagaggacggctgctcctgccggtttcccgaggaagaagaggggggctgcgagctctaa

SEQ ID NO: 4 - protein, 42 aa, human
KRGRKKLLYIFKQPFMRPVQTTQEEDGCSCRFPEEEEGGCEL

SEQ ID NO: 5 - DNA, 81 bp, human
attatctcattcttcctggccctgacctctaccgccctgctgtttctgctgttctttctgaccctgcggttcagcgtcgtg

SEQ ID NO: 6 - protein, 27 aa, human
IISFFLALTSTALLFLLFFLTLRFSVV

SEQ ID NO: 7 - DNA, 78 bp, human
ttccagacactggtcgtgggagtcgtgggcggcctgctgggatctctggtgctgctcgtgtgggtgctggccgtgatc

SEQ ID NO: 8 - protein, 26 aa, human
FQTLVVGVVGGLLGSLVLLVWVLAVI

SEQ ID NO: 9 - DNA, 866 bp, human
atgcagatcccacaggcgccctggccagtcgtctgggcggtgctacaactgggctggcggccaggatggttcttagactccccagacaggccctggaacccccccaccttctccccagccctgctcgtggtgaccgaaggggacaacgccaccttcacctgcagcttctccaacacatcggagagcttcgtgctaaactggtaccgcatgagccccagcaaccagacggacaagctggccgccttccccgaggaccgcagccagcccggccaggactgccgcttccgtgtcacacaactgcccaacgggcgtgacttccacatgagcgtggtcagggcccggcgcaatgacagcggcacctacctctgtggggccatctccctggcccccaaggcgcagatcaaagagagcctgcgggcagagctcagggtgacagagagaagggcagaagtgcccacagcccaccccagcccctcacccaggccagccggccagttccaaaccctggtggttggtgtcgtgggcggcctgctgggcagcctggtgctgctagtctgggtcctggccgtcatctgctcccgggccgcacgagggacaataggagccaggcgcaccggccagcccctgaaggaggacccctcagccgtgcctgtgttctctgtggactatggggagctggatttccagtggcgagagaagaccccggagccccccgtgccctgtgtccctgagcagacggagtatgccaccattgtctttcctagcggaatgggcacctcatcccccgcccgcaggggctcagctgacggccctcggagtgcccagccactgggcctgaggatggacactgctcttggcccctctga

SEQ ID NO: 10 - protein, 288 aa, human
MQIPQAPWPVVWAVLQLGWRPGWFLDSPDRPWNPPTFSPALLVVTEGDNATFTCSFSNTSESFVLNWYRMSPSNQTDKLAAFPEDRSQPGQDCRFRVTQLPNGRDFHMSVVRARRNDSGTYLCGAISLAPKAQIKESLRAELRVTERRAEVPTAHPSPSPRPAGQFQTLVVGVVGGLLGSLVLLVWVLAVICSRAARGTIGARRTGQPLKEDPSAVPVFSVDYGELDFQWREKTPEPPVPCVPEQTEYATIVFPSGMGTSSPARRGSADGPRSAQPLRPEDGHCSWPL

SEQ ID NO: 11 - DNA, 768 bp, human
atgggaaacagctgttacaacatagtagccactctgttgctggtcctcaactttgagaggacaagatcattgcaggatccttgtagtaactgcccagctggtacattctgtgataataacaggaatcagatttgcagtccctgtcctccaaatagtttctccagcgcaggtggacaaaggacctgtgacatatgcaggcagtgtaaaggtgttttcaggaccaggaaggagtgttcctccaccagcaatgcagagtgtgactgcactccagggtttcactgcctgggggcaggatgcagcatgtgtgaacaggattgtaaacaaggtcaagaactgacaaaaaaaggttgtaaagactgttgctttgggacatttaacgatcagaaacgtggcatctgtcgaccctggacaaactgttctttggatggaaagtctgtgcttgtgaatgggacgaaggagagggacgtggtctgtggaccatctccagccgacctctctccgggagcatcctctgtgaccccgcctgcccctgcgagagagccaggacactctccgcagatcatctccttctttcttgcgctgacgtcgactgcgttgctcttcctgctgttcttcctcacgctccgtttctctgttgttaaacggggcagaaagaaactcctgtatatattcaaacaaccatttatgagaccagtacaaactactcaagaggaagatggctgtagctgccgatttccagaagaagaagaaggaggatgtgaactgtga

SEQ ID NO: 12 - protein, 255 aa, human
MGNSCYNIVATLLLVLNFERTRSLQDPCSNCPAGTFCDNNRNQICSPCPPNSFSSAGGQRTCDICRQCKGVFRTRKECSSTSNAECDCTPGFHCLGAGCSMCEQDCKQGQELTKKGCKDCCFGTFNDQKRGICRPWTNCSLDGKSVLVNGTKERDVVCGPSPADLSPGASSVTPPAPAREPGHSPQIISFFLALTSTALLFLLFFLTLRFSVVKRGRKKLLYIFKQPFMRPVQTTQEEDGCSCRFPEEEEGGCEL

SEQ ID NO: 13 - DNA, 663 bp, human
atgctcaggctgctcttggctctcaacttattcccttcaattcaagtaacaggaaacaagattttggtgaagcagtcgcccatgcttgtagcgtacgacaatgcggtcaaccttagctgcaagtattcctacaatctcttctcaagggagttccgggcatcccttcacaaaggactggatagtgctgtggaagtctgtgttgtatatgggaattactcccagcagcttcaggtttactcaaaaacggggttcaactgtgatgggaaattgggcaatgaatcagtgacattctacctccagaatttgtatgttaaccaaacagatatttacttctgcaaaattgaagttatgtatcctcctccttacctagacaatgagaagagcaatggaaccattatccatgtgaaagggaaacacctttgtccaagtcccctatttcccggaccttctaagcccttttgggtgctggtggtggttggtggagtcctggcttgctatagcttgctagtaacagtggcctttattattttctgggtgaggagtaagaggagcaggctcctgcacagtgactacatgaacatgactccccgccgccccgggcccacccgcaagcattaccagccctatgccccaccacgcgacttcgcagcctatcgctcctga

SEQ ID NO: 14 - protein, 220 aa, human
MLRLLLALNLFPSIQVTGNKILVKQSPMLVAYDNAVNLSCKYSYNLFSREFRASLHKGLDSAVEVCVVYGNYSQQLQVYSKTGFNCDGKLGNESVTFYLQNLYVNQTDIYFCKIEVMYPPPYLDNEKSNGTIIHVKGKHLCPSPLFPGPSKPFWVLVVVGGVLACYSLLVTVAFIIFWVRSKRSRLLHSDYMNMTPRRPGPTRKHYQPYAPPRDFAAYRS

SEQ ID NO: 15 - DNA, 867 bp, murine
atgtgggtccggcaggtaccctggtcattcacttgggctgtgctgcagttgagctggcaatcagggtggcttctagaggtccccaatgggccctggaggtccctcaccttctacccagcctggctcacagtgtcagagggagcaaatgccaccttcacctgcagcttgtccaactggtcggaggatcttatgctgaactggaaccgcctgagtcccagcaaccagactgaaaaacaggccgccttctgtaatggtttgagccaacccgtccaggatgcccgcttccagatcatacagctgcccaacaggcatgacttccacatgaacatccttgacacacggcgcaatgacagtggcatctacctctgtggggccatctccctgcaccccaaggcaaaaatcgaggagagccctggagcagagctcgtggtaacagagagaatcctggagacctcaacaagatatcccagcccctcgcccaaaccagaaggccggtttcaaggcatggtcattggtatcatgagtgccctagtgggtatccctgtattgctgctgctggcctgggccctagctgtcttctgctcaacaagtatgtcagaggccagaggagctggaagcaaggacgacactctgaaggaggagccttcagcagcacctgtccctagtgtggcctatgaggagctggacttccagggacgagagaagacaccagagctccctaccgcctgtgtgcacacagaatatgccaccattgtcttcactgaagggctgggtgcctcggccatgggacgtaggggctcagctgatggcctgcagggtcctcggcctccaagacatgaggatggacattgttcttggcctctttga

SEQ ID NO: 16 - protein, 288 aa, murine
MWVRQVPWSFTWAVLQLSWQSGWLLEVPNGPWRSLTFYPAWLTVSEGANATFTCSLSNWSEDLMLNWNRLSPSNQTEKQAAFCNGLSQPVQDARFQIIQLPNRHDFHMNILDTRRNDSGIYLCGAISLHPKAKIEESPGAELVVTERILETSTRYPSPSPKPEGRFQGMVIGIMSALVGIPVLLLLAWALAVFCSTSMSEARGAGSKDDTLKEEPSAAPVPSVAYEELDFQGREKTPELPTACVHTEYATIVFTEGLGASAMGRRGSADGLQGPRPPRHEDGHCSWPL

SEQ ID NO: 17 - DNA, 651 bp, murine
atgggaaacaactgttacaacgtggtggtcattgtgctgctgctagtgggctgtgagaaggtgggagccgtgcagaactcctgtgataactgtcagcctggtactttctgcagaaaatacaatccagtctgcaagagctgccctccaagtaccttctccagcataggtggacagccgaactgtaacatctgcagagtgtgtgcaggctatttcaggttcaagaagttttgctcctctacccacaacgcggagtgtgagtgcattgaaggattccattgcttggggccacagtgcaccagatgtgaaaaggactgcaggcctggccaggagctaacgaagcagggttgcaaaacctgtagcttgggaacatttaatgaccagaacggtactggcgtctgtcgaccctggacgaactgctctctagacggaaggtctgtgcttaagaccgggaccacggagaaggacgtgggaggaccaggagggcactccttgcaggtccttaccttgttcctggcgctgacatcggcttaattcccccacatattcaagcaaccatttaagaagaccactggagcagctcaagaggaagatgcttgtagctgccgatgtccacaggaagaagaaggaggaggaggaggctatgagctgtga

SEQ ID NO: 18 - protein, 256 aa, murine
MGNNCYNVVVIVLLLVGCEKVGAVQNSCDNCQPGTFCRKYNPVCKSCPPSTFSSIGGQPNCNICRVCAGYFRFKKFCSSTHNAECECIEGFHCLGPQCTRCEKDCRPGQELTKQGCKTCSLGTFNDQNGTGVCRPWTNCSLDGRSVLKTGTTEKDVVCGPPVVSFSPSTTISVTPEGGPGGHSLQVLTLFLALTSALLLALIFITLLFSVLKWIRKKFPHIFKQPFKKTTGAAQEEDACSCRCPQEEEGGGGGYEL

SEQ ID NO: 19 - DNA, 657 bp, murine
atgacactcaggctgctgttcttggctctcaacttcttctcagttcaagtaacagaaaacaagattttggtaaagcagtcgcccctgcttgtggtagatagcaacgaggtcagcctcagctgcaggtattcctacaaccttctcgcaaaggaattccgggcatccctgtacaagggcgtgaacagcgacgtggaagtctgtgtcgggaatgggaattttacctatcagccccagtttcgctcgaatgccgagttcaactgcgacggggatttcgacaacgaaacagtgacgttccgtctctggaatctgcacgtcaatcacacagatatttacttctgcaaaattgagttcatgtaccctccgccttacctagacaacgagaggagcaatggaactattattcacataaaagagaaacatctttgtcatactcagtcatctcctaagctgttttgggcactggtcgtggttgctggagtcctgttttgttatggcttgctagtgacagtggctctttgtgttatctggacaaatagtagaaggaacagactccttcaagtgactaccatgaacatgactccccggaggcctgggctcactcgaaagccttaccagccctacgcccctgccagagactttgcagcgtaccgcccctga

SEQ ID NO: 20 - protein, 218 aa, murine
MTLRLLFLALNFFSVQVTENKILVKQSPLLVVDSNEVSLSCRYSYNLLAKEFRASLYKGVNSDVEVCVGNGNFTYQPQFRSNAEFNCDGDFDNETVTFRLWNLHVNHTDIYFCKIEFMYPPPYLDNERSNGTIIHIKEKHLCHTQSSPKLFWALVVVAGVLFCYGLLVTVALCVIWTNSRRNRLLQVTTMNMTPRRPGLTRKPYQPYAPARDFAAYRP

SEQ ID NO: 21 - DNA, 705 bp, human
atgcagattcctcaggccccttggcctgtcgtgtgggctgtgctccagctgggatggcggcctggctggtttctggacagccccgacagaccctggaacccccctacattttcccctgccctgctggtcgtgaccgagggcgacaatgccaccttcacctgtagcttcagcaacaccagcgagagcttcgtgctgaactggtacagaatgagccccagcaaccagaccgacaagctggccgccttccccgaggatagatctcagcccggccaggactgccggttcagagtgacccagctgcccaacggccgggacttccacatgtctgtcgtgcgggccagacggaacgacagcggcacatatctgtgcggcgccatcagcctggcccccaaggcccagatcaaagagagcctgagagccgagctgagagtgaccgagagaagggccgaagtgcctaccgcccaccctagcccatctccaagacctgccggccagattatctcattcttcctggccctgacctctaccgccctgctgtttctgctgttctttctgaccctgcggttcagcgtcgtgaagcggggcagaaagaagctgctgtacatcttcaagcagcccttcatgcggcccgtgcagaccacccaggaagaggacggctgctcctgccggtttcccgaggaagaagaggggggctgcgagctctaa

SEQ ID NO: 22 - protein, 230 aa, human
MQIPQAPWPVVWAVLQLGWRPGWFLDSPDRPWNPPTFSPALLVVTEGDNATFTCSFSNTSESFVLNWYRMSPSNQTDKLAAFPEDRSQPGQDCRFRVTQLPNGRDFHMSVVRARRNDSGTYLCGAISLAPKAQIKESLRAELRVTERRAEVPTAHPSPSPRPAGQIISFFLALTSTALLFLLFFLTLRFSVVKRGRKKLLYIFKQPFMRPVQTTQEEDGCSCRFPEEEEG

SEQ ID NO: 23 - DNA, 702 bp, human
atgcagattcctcaggctccttggcctgtcgtgtgggccgtgctccagctgggatggcggcctggatggttcctggacagccccgacagaccctggaacccccctacattttcccctgccctgctggtcgtgaccgagggcgacaatgccaccttcacctgtagcttcagcaacaccagcgagagcttcgtgctgaactggtacagaatgagccccagcaaccagaccgacaagctggccgccttccccgaggatagatctcagcccggccaggactgccggttcagagtgacccagctgcccaacggccgggacttccacatgtctgtcgtgcgcgccagacggaacgacagcggcacatatctgtgcggcgccatcagcctggcccccaaggcccagatcaaagagagcctgagagccgagctgagagtgaccgagagaagggccgaagtgcctaccgcccaccctagcccatctccaagacctgccggccagttccagacactggtcgtgggagtcgtgggcggcctgctgggatctctggtgctgctcgtgtgggtgctggccgtgatcaagcggggcagaaagaagctgctgtacatcttcaagcagcccttcatgcggcccgtgcagaccacccaggaagaggacggctgctcctgccggtttcccgaggaagaagaggggggctgcgagctctaa

SEQ ID NO: 24 - protein, 230 aa, human
MQIPQAPWPVVWAVLQLGWRPGWFLDSPDRPWNPPTFSPALLVVTEGDNATFTCSFSNTSESFVLNWYRMSPSNQTDKLAAFPEDRSQPGQDCRFRVTQLPNGRDFHMSVVRARRNDSGTYLCGAISLAPKAQIKESLRAELRVTERRAEVPTAHPSPSPRPAGQFQTLVVGVVGGLLGSLVLLVWVLAVIKRGRKKLLYIFKQPFMRPVQTTQEEDGCSCRFPEEEEGG

SEQ ID NO: 25 - DNA, 702 bp, human
atgcagattcctcaggccccttggcctgtcgtgtgggctgtgctccagctgggatggcggcctggctggtttctggacagccccgacagaccctggaacccccctacattttcccctgccctgctggtcgtgaccgagggcgacaatgccaccttcacctgtagcttcagcaacaccagcgagagcttcgtgctgaactggtacagaatgagccccagcaaccagaccgacaagctggccgccttccccgaggatagatctcagcccggccaggattgccggttcagagtgacccagctgcccaacggccgggacttccacatgtctgtcgtgcgggccagacggaacgacagcggcacatatctgtgcggcgccatcagcctggcccccaaggcccagatcaaagagagcctgagagccgagctgagagtgaccgagagaagggccgaagtgcctaccgcccaccctagcccatctccaagacctgccggccagttctgggtgctggtggtcgtgggcggagtgctggcctgttacagcctgctcgtgaccgtggccttcatcatcttttgggtgcgcagcaagcggagccggctgctgcacagcgactacatgaacatgacccccagacggccaggccccaccagaaagcactaccagccttacgcccctcccagagacttcgccgcctacagaagctga

SEQ ID NO: 26 - protein, 233 aa, human
MQIPQAPWPVVWAVLQLGWRPGWFLDSPDRPWNPPTFSPALLVVTEGDNATFTCSFSNTSESFVLNWYRMSPSNQTDKLAAFPEDRSQPGQDCRFRVTQLPNGRDFHMSVVRARRNDSGTYLCGAISLAPKAQIKESLRAELRVTERRAEVPTAHPSPSPRPAGQFWVLVVVGGVLACYSLLVTVAFIIFWVRSKRSRLLHSDYMNMTPRRPGPTRKHYQPYAPPRDFAAYRS

SEQ ID NO: 27 - protein, 483 aa, human
MQIPQAPWPVVWAVLQLGWRMQKGDQNPQIAAHVISEASSKTTSVLQWAEKGYYTMSNNLVTLENGKQLTVKRQGLYYIYAQVTFCSNREASSQAPFIASLCLKSPGRFERILLRAANTHSSAKPCGQQSIHLGGVFELQPGASVFVNVTDPSQVSHGTGFTSFGLLKLGGGGSGGGGDEPKSCDKTHTCPPCPAPPVAGPSVFLFPPKPKDTLMIARTPEVTCVVVDVSHEDPEVKFNWYVDGVEVHNAKTKPREEQYNSTYRVVSVLTVLHQDWLNGKEYKCKVSNKALPAPIEKTISKAKGQPREPQVYTLPPSRDELTKNQVSLTCLVKGFYPSDIAVEWESNGQPENNYKTTPPVLDSDGSFFLYSKLTVDKSRWQQGNVFSCSVMHEALHNHYTQKSLSLSPGKGPSKPFWVLVVVGGVLACYSLLVTVAFIIFWVRSKRSRLLHSDYMNMTPRRPGPTRKHYQPYAPPRDFAAYRS

SEQ ID NO: 28 - protein, 348 aa, human
MQIPQAPWPVVWAVLQLGWRMQKGDQNPQIAAHVISEASSKTTSVLQWAEKGYYTMSNNLVTLENGKQLTVKRQGLYYIYAQVTFCSNREASSQAPFIASLCLKSPGRFERILLRAANTHSSAKPCGQQSIHLGGVFELQPGASVFVNVTDPSQVSHGTGFTSFGLLKLGGGGSGGGGDGQACNPSACRAVGRGLQPKGVRVKETADFKVYTKGAGSGELKVTVKGPKGEERVKQKDLGDGVYGFEYYPMVPGTYIVTITWGGQNIGRSPFEVKVGPSKPFWVLVVVGGVLACYSLLVTVAFIIFWVRSKRSRLLHSDYMNMTPRRPGPTRKHYQPYAPPRDFAAYRS

SEQ ID NO: 29 - protein, 290 aa, human
MRSKRSRLLHSDYMNMTPRRPGPTRKHYQPYAPPRDFAAYRSATGLPISMKIFMYLLTVFLITQMIGSALFAVYLHRRLDKIEDERNLHEDFVFMKTIQRCNTGERSLSLLNCEEIKSQFEGFVKDIMLNKEETKKENSFEMQKGDQNPQIAAHVISEASSKTTSVLQWAEKGYYTMSNNLVTLENGKQLTVKRQGLYYIYAQVTFCSNREASSQAPFIASLCLKSPGRFERILLRAANTHSSAKPCGQQSIHLGGVFELQPGASVFVNVTDPSQVSHGTGFTSFGLLKL

SEQ ID NO: 30 - protein, 261 aa, human
MIETYNQTSPRSAATGLPISMKIFMYLLTVFLITQMIGSALFAVYLHRRLDKIEDERNLHEDFVFMKTIQRCNTGERSLSLLNCEEIKSQFEGFVKDIMLNKEETKKENSFEMQKGDQNPQIAAHVISEASSKTTSVLQWAEKGYYTMSNNLVTLENGKQLTVKRQGLYYIYAQVTFCSNREASSQAPFIASLCLKSPGRFERILLRAANTHSSAKPCGQQSIHLGGVFELQPGASVFVNVTDPSQVSHGTGFTSFGLLKL